European Patent Application EP 4 425 181 A1, published September 4, 2024. Title: Composition for detecting or measuring analytes. Applicant: BERTIS Inc. Application EP. The sequence listing filed with the application follows.

SEQUENCE LISTING (691 sequences)

SEQ ID NO: 1 - protein, 6 aa, synthetic construct
  REGION 1..6: note = peptide
LNHEGK

SEQ ID NO: 2 - protein, 8 aa, synthetic construct
  REGION 1..8: note = peptide
AAATNPAR

SEQ ID NO: 3 - protein, 7 aa, synthetic construct
  REGION 1..7: note = peptide
SPEDEEK

SEQ ID NO: 4 - protein, 7 aa, synthetic construct
  REGION 1..7: note = peptide
EGGHNIK

SEQ ID NO: 5 - protein, 7 aa, synthetic construct
  REGION 1..7: note = peptide
NAGPTAR

SEQ ID NO: 6 - protein, 7 aa, synthetic construct
  REGION 1..7: note = peptide
FSNSGSR

SEQ ID NO: 7 - protein, 9 aa, synthetic construct
  REGION 1..9: note = peptide
NDSEPGSQR

SEQ ID NO: 8 - protein, 7 aa, synthetic construct
  REGION 1..7: note = peptide
TGVIHEK

SEQ ID NO: 9 - protein, 8 aa, synthetic construct
  REGION 1..8: note = peptide
LVHHNVTR

SEQ ID NO: 10 - protein, 10 aa, synthetic construct
  REGION 1..10: note = peptide
THHDGAITER

SEQ ID NO: 11 - protein, 6 aa, synthetic construct
  REGION 1..6: note = peptide
WTNQQK

SEQ ID NO: 12 - protein, 7 aa, synthetic construct
  REGION 1..7: note = peptide
VNDSGYK

SEQ ID NO: 13 - protein, 7 aa, synthetic construct
  REGION 1..7: note = peptide
VGSDTVR

SEQ ID NO: 14 - protein, 6 aa, synthetic construct
  REGION 1..6: note = peptide
VSQALR

SEQ ID NO: 15 - protein, 7 aa, synthetic construct
  REGION 1..7: note = peptide
ENGTISR

SEQ ID NO: 16 - protein, 7 aa, synthetic construct
  REGION 1..7: note = peptide
SVDGPIR

SEQ ID NO: 17 - protein, 6 aa, synthetic construct
  REGION 1..6: note = peptide
FTEPSR

SEQ ID NO: 18 - protein, 7 aa, synthetic construct
  REGION 1..7: note = peptide
ETFGDSK

SEQ ID NO: 19 - protein, 5 aa, synthetic construct
  REGION 1..5: note = peptide
HSPGR

SEQ ID NO: 20 - protein, 5 aa, synthetic construct
  REGION 1..5: note = peptide
NGVHK

SEQ ID NO: 21 - protein, 7 aa, synthetic construct
  REGION 1..7: note = peptide
NNFGNGR

SEQ ID NO: 22 - protein, 8 aa, synthetic construct
  REGION 1..8: note = peptide
GDSTFESK

SEQ ID NO: 23 - protein, 10 aa, synthetic construct
  REGION 1..10: note = peptide
EEQEETSAIR

SEQ ID NO: 24 - protein, 9 aa, synthetic construct
  REGION 1..9: note = peptide
FQEGQEEER

SEQ ID NO: 25 - protein, 7 aa, synthetic construct
  REGION 1..7: note = peptide
ILDGGNK

SEQ ID NO: 26 - protein, 5 aa, synthetic construct
  REGION 1..5: note = peptide
TQTPK

SEQ ID NO: 27 - protein, 7 aa, synthetic construct
  REGION 1..7: note = peptide
VAHLTGK

SEQ ID NO: 28 - protein, 7 aa, synthetic construct
  REGION 1..7: note = peptide
VLVEQTK

SEQ ID NO: 29 - protein, 5 aa, synthetic construct
  REGION 1..5: note = peptide
FDGHR

SEQ ID NO: 30 - protein, 7 aa, synthetic construct
  REGION 1..7: note = peptide
YHEEFEK

SEQ ID NO: 31 - protein, 8 aa, synthetic construct
  REGION 1..8: note = peptide
SDFSNEER

SEQ ID NO: 32 - protein, 6 aa, synthetic construct
  REGION 1..6: note = peptide
ATAGFR

SEQ ID NO: 33 - protein, 7 aa, synthetic construct
  REGION 1..7: note = peptide
LHGTLPK

SEQ ID NO: 34 - protein, 8 aa, synthetic construct
  REGION 1..8: note = peptide
SGSGLVGR

SEQ ID NO: 35 - protein, 8 aa, synthetic construct
  REGION 1..8: note = peptide
AVLIPHHK

SEQ ID NO: 36 - protein, 10 aa, synthetic construct
  REGION 1..10: note = peptide
SQLANTEPTK

SEQ ID NO: 37 - protein, 6 aa, synthetic construct
  REGION 1..6: note = peptide
WQHQIK

SEQ ID NO: 38 - protein, 8 aa, synthetic construct
  REGION 1..8: note = peptide
LIAQASEK

SEQ ID NO: 39 - protein, 8 aa, synthetic construct
  REGION 1..8: note = peptide
VAQELEEK

SEQ ID NO: 40 - protein, 8 aa, synthetic construct
  REGION 1..8: note = peptide
EQAALVSK

SEQ ID NO: 41 - protein, 12 aa, synthetic construct
  REGION 1..12: note = peptide
YVPNSGQEDADR

SEQ ID NO: 42 - protein, 9 aa, synthetic construct
  REGION 1..9: note = peptide
SADSHGHPR

SEQ ID NO: 43 - protein, 5 aa, synthetic construct
  REGION 1..5: note = peptide
ISPDR

SEQ ID NO: 44 - protein, 8 aa, synthetic construct
  REGION 1..8: note = peptide
ASLAEETR

SEQ ID NO: 45 - protein, 7 aa, synthetic construct
  REGION 1..7: note = peptide
NGNFHPK

SEQ ID NO: 46 - protein, 6 aa, synthetic construct
  REGION 1..6: note = peptide
LYVVEK

SEQ ID NO: 47 - protein, 9 aa, synthetic construct
  REGION 1..9: note = peptide
FVTQAEGAK

SEQ ID NO: 48 - protein, 11 aa, synthetic construct
  REGION 1..11: note = peptide
GSQGAIPPPDK

SEQ ID NO: 49 - protein, 8 aa, synthetic construct
  REGION 1..8: note = peptide
IQGDLAGR

SEQ ID NO: 50 - protein, 6 aa, synthetic construct
  REGION 1..6: note = peptide
SVETIK

SEQ ID NO: 51 - protein, 5 aa, synthetic construct
  REGION 1..5: note = peptide
TIVAK

SEQ ID NO: 52 - protein, 7 aa, synthetic construct
  REGION 1..7: note = peptide
SHTALLR

SEQ ID NO: 53 - protein, 8 aa, synthetic construct
  REGION 1..8: note = peptide
SSDANLYR

SEQ ID NO: 54 - protein, 7 aa, synthetic construct
  REGION 1..7: note = peptide
ELVHTYK

SEQ ID NO: 55 - protein, 5 aa, synthetic construct
  REGION 1..5: note = peptide
GNVLR

SEQ ID NO: 56 - protein, 5 aa, synthetic construct
  REGION 1..5: note = peptide
DDVIK

SEQ ID NO: 57 - protein, 8 aa, synthetic construct
  REGION 1..8: note = peptide
EVFEDSDK

SEQ ID NO: 58 - protein, 8 aa, synthetic construct
  REGION 1..8: note = peptide
ILADATAK

SEQ ID NO: 59 - protein, 10 aa, synthetic construct
  REGION 1..10: note = peptide
IAGDQSTLQR

SEQ ID NO: 60 - protein, 9 aa, synthetic construct
  REGION 1..9: note = peptide
GEAGVIGER

SEQ ID NO: 61 - protein, 8 aa, synthetic construct
  REGION 1..8: note = peptide
ITQDAQLK

SEQ ID NO: 62 - protein, 8 aa, synthetic construct
  REGION 1..8: note = peptide
TQVEELSK

SEQ ID NO: 63 - protein, 8 aa, synthetic construct
  REGION 1..8: note = peptide
GGVASGFK

SEQ ID NO: 64 - protein, 7 aa, synthetic construct
  REGION 1..7: note = peptide
GAAFVSK

SEQ ID NO: 65 - protein, 7 aa, synthetic construct
  REGION 1..7: note = peptide
IQTQLQR

SEQ ID NO: 66 - protein, 11 aa, synthetic construct
  REGION 1..11: note = peptide
IQGDGAALQEK

SEQ ID NO: 67 - protein, 6 aa, synthetic construct
  REGION 1..6: note = peptide
YIGVGK

SEQ ID NO: 68 - protein, 8 aa, synthetic construct
  REGION 1..8: note = peptide
FPSTSESR

SEQ ID NO: 69 - protein, 8 aa, synthetic construct
  REGION 1..8: note = peptide
LNVEGTER

SEQ ID NO: 70 - protein, 11 aa, synthetic construct
  REGION 1..11: note = peptide
SSALQVSGSTR

SEQ ID NO: 71 - protein, 8 aa, synthetic construct
  REGION 1..8: note = peptide
EVFENTER

SEQ ID NO: 72 - protein, 7 aa, synthetic construct
  REGION 1..7: note = peptide
DGPEQLR

SEQ ID NO: 73 - protein, 6 aa, synthetic construct
  REGION 1..6: note = peptide
VAEAFR

SEQ ID NO: 74 - protein, 9 aa, synthetic construct
  REGION 1..9: note = peptide
QAFQGAVQK

SEQ ID NO: 75 - protein, 7 aa, synthetic construct
  REGION 1..7: note = peptide
SLGDLEK

SEQ ID NO: 76 - protein, 8 aa, synthetic construct
  REGION 1..8: note = peptide
EVATEGIR

SEQ ID NO: 77 - protein, 7 aa, synthetic construct
  REGION 1..7: note = peptide
VPPEDIK

SEQ ID NO: 78 - protein, 9 aa, synthetic construct
  REGION 1..9: note = peptide
ATVVYQGER

SEQ ID NO: 79 - protein, 6 aa, synthetic construct
  REGION 1..6: note = peptide
VGDVLK

SEQ ID NO: 80 - protein, 11 aa, synthetic construct
  REGION 1..11: note = peptide
LSSTTTTTGLR

SEQ ID NO: 81 - protein, 8 aa, synthetic construct
  REGION 1..8: note = peptide
QVFGEATK

SEQ ID NO: 82 - protein, 8 aa, synthetic construct
  REGION 1..8: note = peptide
SDIAPVAR

SEQ ID NO: 83 - protein, 10 aa, synthetic construct
  REGION 1..10: note = peptide
GISSTTVTGR

SEQ ID NO: 84 - protein, 10 aa, synthetic construct
  REGION 1..10: note = peptide
TAATAALAGR

SEQ ID NO: 85 - protein, 5 aa, synthetic construct
  REGION 1..5: note = peptide
FPDGR

SEQ ID NO: 86 - protein, 6 aa, synthetic construct
  REGION 1..6: note = peptide
QVPLQR

SEQ ID NO: 87 - protein, 11 aa, synthetic construct
  REGION 1..11: note = peptide
DADSINSSIDK

SEQ ID NO: 88 - protein, 8 aa, synthetic construct
  REGION 1..8: note = peptide
ELGYVEAK

SEQ ID NO: 89 - protein, 6 aa, synthetic construct
  REGION 1..6: note = peptide
VDPHFR

SEQ ID NO: 90 - protein, 8 aa, synthetic construct
  REGION 1..8: note = peptide
VILDGGDR

SEQ ID NO: 91 - protein, 8 aa, synthetic construct
  REGION 1..8: note = peptide
AGVGQSWK

SEQ ID NO: 92 - protein, 7 aa, synthetic construct
  REGION 1..7: note = peptide
TDQYWEK

SEQ ID NO: 93 - protein, 8 aa, synthetic construct
  REGION 1..8: note = peptide
LTWASHEK

SEQ ID NO: 94 - protein, 7 aa, synthetic construct
  REGION 1..7: note = peptide
VQDVIER

SEQ ID NO: 95 - protein, 8 aa, synthetic construct
  REGION 1..8: note = peptide
SGDFYTEK

SEQ ID NO: 96 - protein, 8 aa, synthetic construct
  REGION 1..8: note = peptide
DQVETALK

SEQ ID NO: 97 - protein, 9 aa, synthetic construct
  REGION 1..9: note = peptide
SSQAGIPVR

SEQ ID NO: 98 - protein, 10 aa, synthetic construct
  REGION 1..10: note = peptide
VYSTSVTGSR

SEQ ID NO: 99 - protein, 10 aa, synthetic construct
  REGION 1..10: note = peptide
STTPASNIVR

SEQ ID NO: 100 - protein, 5 aa, synthetic construct
  REGION 1..5: note = peptide
ADIIR

SEQ ID NO: 101 - protein, 10 aa, synthetic construct
  REGION 1..10: note = peptide
TTSDGGYSFK

SEQ ID NO: 102 - protein, 10 aa, synthetic construct
  REGION 1..10: note = peptide
VFQQVAQASK

SEQ ID NO: 103 - protein, 5 aa, synthetic construct
  REGION 1..5: note = peptide
ALVVK

SEQ ID NO: 104 - protein, 8 aa, synthetic construct
  REGION 1..8: note = peptide
EAFAAVSK

SEQ ID NO: 105 - protein, 9 aa, synthetic construct
  REGION 1..9: note = peptide
EDGSVDFQR

SEQ ID NO: 106 - protein, 8 aa, synthetic construct
  REGION 1..8: note = peptide
VTFEESAK

SEQ ID NO: 107 - protein, 5 aa, synthetic construct
  REGION 1..5: note = peptide
IPIQR

SEQ ID NO: 108 - protein, 8 aa, synthetic construct
  REGION 1..8: note = peptide
SSSISSFK

SEQ ID NO: 109 - protein, 11 aa, synthetic construct
  REGION 1..11: note = peptide
DLVVQQAGTNK

SEQ ID NO: 110 - protein, 8 aa, synthetic construct
  REGION 1..8: note = peptide
LPGAHLQR

SEQ ID NO: 111 - protein, 7 aa, synthetic construct
  REGION 1..7: note = peptide
AHLTVVR

SEQ ID NO: 112 - protein, 8 aa, synthetic construct
  REGION 1..8: note = peptide
QYTDSTFR

SEQ ID NO: 113 - protein, 12 aa, synthetic construct
  REGION 1..12: note = peptide
DGHSESSTLIGR

SEQ ID NO: 114 - protein, 8 aa, synthetic construct
  REGION 1..8: note = peptide
QLTPYAQR

SEQ ID NO: 115 - protein, 10 aa, synthetic construct
  REGION 1..10: note = peptide
GSGLSLASGR

SEQ ID NO: 116 - protein, 8 aa, synthetic construct
  REGION 1..8: note = peptide
ELGFGSAK

SEQ ID NO: 117 - protein, 8 aa, synthetic construct
  REGION 1..8: note = peptide
VTVLGQPK

SEQ ID NO: 118 - protein, 6 aa, synthetic construct
  REGION 1..6: note = peptide
VAGWGR

SEQ ID NO: 119 - protein, 5 aa, synthetic construct
  REGION 1..5: note = peptide
QTWVK

SEQ ID NO: 120 - protein, 15 aa, synthetic construct
  REGION 1..15: note = peptide
TAGGGPDSELQPQDK

SEQ ID NO: 121 - protein, 11 aa, synthetic construct
  REGION 1..11: note = peptide
YSPGGTPTAIK

SEQ ID NO: 122 - protein, 11 aa, synthetic construct
  REGION 1..11: note = peptide
QHADAVHLISR

SEQ ID NO: 123 - protein, 9 aa, synthetic construct
  REGION 1..9: note = peptide
LEPQAAVVK

SEQ ID NO: 124 - protein, 7 aa, synthetic construct
  REGION 1..7: note = peptide
TLLTAAR

SEQ ID NO: 125 - protein, 9 aa, synthetic construct
  REGION 1..9: note = peptide
LTEATQLGK

SEQ ID NO: 126 - protein, 5 aa, synthetic construct
  REGION 1..5: note = peptide
SYFEK

SEQ ID NO: 127 - protein, 7 aa, synthetic construct
  REGION 1..7: note = peptide
AILSTYR

SEQ ID NO: 128 - protein, 6 aa, synthetic construct
  REGION 1..6: note = peptide
SPYGFR

SEQ ID NO: 129 - protein, 9 aa, synthetic construct
  REGION 1..9: note = peptide
VLIAHNQVR

SEQ ID NO: 130 - protein, 9 aa, synthetic construct
  REGION 1..9: note = peptide
VVSYQLSSR

SEQ ID NO: 131 - protein, 8 aa, synthetic construct
  REGION 1..8: note = peptide
IPGSPEIR

SEQ ID NO: 132 - protein, 10 aa, synthetic construct
  REGION 1..10: note = peptide
AEQSLQAAIK

SEQ ID NO: 133 - protein, 12 aa, synthetic construct
  REGION 1..12: note = peptide
SVNAQVTDINSK

SEQ ID NO: 134 - protein, 8 aa, synthetic construct
  REGION 1..8: note = peptide
ASSFLGEK

SEQ ID NO: 135 - protein, 8 aa, synthetic construct
  REGION 1..8: note = peptide
DEQVPFSK

SEQ ID NO: 136 - protein, 9 aa, synthetic construct
  REGION 1..9: note = peptide
ESGVLLTDK

SEQ ID NO: 137 - protein, 6 aa, synthetic construct
  REGION 1..6: note = peptide
EGYLVK

SEQ ID NO: 138 - protein, 6 aa, synthetic construct
  REGION 1..6: note = peptide
SVEVLK

SEQ ID NO: 139 - protein, 8 aa, synthetic construct
  REGION 1..8: note = peptide
ALEQALEK

SEQ ID NO: 140 - protein, 6 aa, synthetic construct
  REGION 1..6: note = peptide
QWQTLK

SEQ ID NO: 141 - protein, 9 aa, synthetic construct
  REGION 1..9: note = peptide
DALSASVVK

SEQ ID NO: 142 - protein, 7 aa, synthetic construct
  REGION 1..7: note = peptide
VDPVNFK

SEQ ID NO: 143 - protein, 9 aa, synthetic construct
  REGION 1..9: note = peptide
DGSTIPIAK

SEQ ID NO: 144 - protein, 10 aa, synthetic construct
  REGION 1..10: note = peptide
FDDESAEEIR

SEQ ID NO: 145 - protein, 11 aa, synthetic construct
  REGION 1..11: note = peptide
TNDPGVLQAAR

SEQ ID NO: 146 - protein, 10 aa, synthetic construct
  REGION 1..10: note = peptide
EGTEASLQIR

SEQ ID NO: 147 - protein, 7 aa, synthetic construct
  REGION 1..7: note = peptide
GGVLIQR

SEQ ID NO: 148 - protein, 9 aa, synthetic construct
  REGION 1..9: note = peptide
ALNSVAYER

SEQ ID NO: 149 - protein, 9 aa, synthetic construct
  REGION 1..9: note = peptide
LTQGDYFTK

SEQ ID NO: 150 - protein, 8 aa, synthetic construct
  REGION 1..8: note = peptide
AGLSTVYK

SEQ ID NO: 151 - protein, 11 aa, synthetic construct
  REGION 1..11: note = peptide
LFDASDSSSYK

SEQ ID NO: 152 - protein, 8 aa, synthetic construct
  REGION 1..8: note = peptide
VGVNGFGR

SEQ ID NO: 153 - protein, 9 aa, synthetic construct
  REGION 1..9: note = peptide
GPGGVWAAK

SEQ ID NO: 154 - protein, 9 aa, synthetic construct
  REGION 1..9: note = peptide
YEYLEGGDR

SEQ ID NO: 155 - protein, 10 aa, synthetic construct
  REGION 1..10: note = peptide
YVSALTTPAR

SEQ ID NO: 156 - protein, 7 aa, synthetic construct
  REGION 1..7: note = peptide
SLLQPNK

SEQ ID NO: 157 - protein, 9 aa, synthetic construct
  REGION 1..9: note = peptide
GTPPGVYIK

SEQ ID NO: 158 - protein, 9 aa, synthetic construct
  REGION 1..9: note = peptide
FQASVATPR

SEQ ID NO: 159 - protein, 7 aa, synthetic construct
  REGION 1..7: note = peptide
QVFAVQR

SEQ ID NO: 160 - protein, 8 aa, synthetic construct
  REGION 1..8: note = peptide
EIFGQDAR

SEQ ID NO: 161 - protein, 10 aa, synthetic construct
  REGION 1..10: note = peptide
SVNPYLQGQR

SEQ ID NO: 162 - protein, 10 aa, synthetic construct
  REGION 1..10: note = peptide
GTFSTTVTGR

SEQ ID NO: 163 - protein, 6 aa, synthetic construct
  REGION 1..6: note = peptide
LLSEVR

SEQ ID NO: 164 - protein, 8 aa, synthetic construct
  REGION 1..8: note = peptide
EYFYTSGK

SEQ ID NO: 165 - protein, 9 aa, synthetic construct
  REGION 1..9: note = peptide
AILGATEVK

SEQ ID NO: 166 - protein, 8 aa, synthetic construct
  REGION 1..8: note = peptide
VLDEATLK

SEQ ID NO: 167 - protein, 11 aa, synthetic construct
  REGION 1..11: note = peptide
EQVDQGPDWER

SEQ ID NO: 168 - protein, 9 aa, synthetic construct
  REGION 1..9: note = peptide
DGPDTLLSK

SEQ ID NO: 169 - protein, 7 aa, synthetic construct
  REGION 1..7: note = peptide
GWSPTPR

SEQ ID NO: 170 - protein, 9 aa, synthetic construct
  REGION 1..9: note = peptide
QLYSALANK

SEQ ID NO: 171 - protein, 8 aa, synthetic construct
  REGION 1..8: note = peptide
VSISTLNK

SEQ ID NO: 172 - protein, 8 aa, synthetic construct
  REGION 1..8: note = peptide
DFVQPPTK

SEQ ID NO: 173 - protein, 9 aa, synthetic construct
  REGION 1..9: note = peptide
NAIEALGSK

SEQ ID NO: 174 - protein, 9 aa, synthetic construct
  REGION 1..9: note = peptide
EDGSLDFQR

SEQ ID NO: 175 - protein, 7 aa, synthetic construct
  REGION 1..7: note = peptide
DQLVLGR

SEQ ID NO: 176 - protein, 11 aa, synthetic construct
  REGION 1..11: note = peptide
NANTFISPQQR

SEQ ID NO: 177 - protein, 7 aa, synthetic construct
  REGION 1..7: note = peptide
SPQAFYR

SEQ ID NO: 178 - protein, 10 aa, synthetic construct
  REGION 1..10: note = peptide
SGIIIIAIHR

SEQ ID NO: 179 - protein, 10 aa, synthetic construct
  REGION 1..10: note = peptide
EGSDLSVVER

SEQ ID NO: 180 - protein, 11 aa, synthetic construct
  REGION 1..11: note = peptide
AVEPQLQEEER

SEQ ID NO: 181 - protein, 11 aa, synthetic construct
  REGION 1..11: note = peptide
ISSAGASFGSR

SEQ ID NO: 182 - protein, 5 aa, synthetic construct
  REGION 1..5: note = peptide
AWTYR

SEQ ID NO: 183 - protein, 9 aa, synthetic construct
  REGION 1..9: note = peptide
GGPFSDSYR

SEQ ID NO: 184 - protein, 8 aa, synthetic construct
  REGION 1..8: note = peptide
VTTNPNLR

SEQ ID NO: 185 - protein, 9 aa, synthetic construct
  REGION 1..9: note = peptide
DEVEDDYIK

SEQ ID NO: 186 - protein, 20 aa, synthetic construct
  REGION 1..20: note = peptide
PAPGSTAPPAHGVTSAPDTR

SEQ ID NO: 187 - protein, 7 aa, synthetic construct
  REGION 1..7: note = peptide
NQNTFLR

SEQ ID NO: 188 - protein, 12 aa, synthetic construct
  REGION 1..12: note = peptide
GLGDDTALNDAR

SEQ ID NO: 189 - protein, 5 aa, synthetic construct
  REGION 1..5: note = peptide
LSVIR

SEQ ID NO: 190 - protein, 9 aa, synthetic construct
  REGION 1..9: note = peptide
LIQGAPTIR

SEQ ID NO: 191 - protein, 7 aa, synthetic construct
  REGION 1..7: note = peptide
FPSGTLR

SEQ ID NO: 192 - protein, 9 aa, synthetic construct
  REGION 1..9: note = peptide
EDAVSAAFK

SEQ ID NO: 193 - protein, 8 aa, synthetic construct
  REGION 1..8: note = peptide
VAELEDEK

SEQ ID NO: 194 - protein, 12 aa, synthetic construct
  REGION 1..12: note = peptide
FVGGAENTAHPR

SEQ ID NO: 195 - protein, 13 aa, synthetic construct
  REGION 1..13: note = peptide
EVASNSELVQSSR

SEQ ID NO: 196 - protein, 12 aa, synthetic construct
  REGION 1..12: note = peptide
AAISGENAGLVR

SEQ ID NO: 197 - protein, 9 aa, synthetic construct
  REGION 1..9: note = peptide
TGLQEVEVK

SEQ ID NO: 198 - protein, 9 aa, synthetic construct
  REGION 1..9: note = peptide
TYLPAVDEK

SEQ ID NO: 199 - protein, 8 aa, synthetic construct
  REGION 1..8: note = peptide
GGLVDITR

SEQ ID NO: 200 - protein, 13 aa, synthetic construct
  REGION 1..13: note = peptide
INDISHTQSVSSK

SEQ ID NO: 201 - protein, 6 aa, synthetic construct
  REGION 1..6: note = peptide
FYQDLK

SEQ ID NO: 202 - protein, 7 aa, synthetic construct
  REGION 1..7: note = peptide
VEVLVER

SEQ ID NO: 203 - protein, 9 aa, synthetic construct
  REGION 1..9: note = peptide
LQAEAFQAR

SEQ ID NO: 204 - protein, 10 aa, synthetic construct
  REGION 1..10: note = peptide
AYTGFEQAAR

SEQ ID NO: 205 - protein, 11 aa, synthetic construct
  REGION 1..11: note = peptide
TGQIFNQSYSK

SEQ ID NO: 206 - protein, 11 aa, synthetic construct
  REGION 1..11: note = peptide
HSENFAWTENR

SEQ ID NO: 207 - protein, 8 aa, synthetic construct
  REGION 1..8: note = peptide
ELGFGSAR

SEQ ID NO: 208 - protein, 5 aa, synthetic construct
  REGION 1..5: note = peptide
AVIFK

SEQ ID NO: 209 - protein, 9 aa, synthetic construct
  REGION 1..9: note = peptide
GFVVAGPSR

SEQ ID NO: 210 - protein, 11 aa, synthetic construct
  REGION 1..11: note = peptide
SNFVPTNVGSK

SEQ ID NO: 211 - protein, 9 aa, synthetic construct
  REGION 1..9: note = peptide
SLVGLGGTK

SEQ ID NO: 212 - protein, 9 aa, synthetic construct
  REGION 1..9: note = peptide
VSVYAVPDK

SEQ ID NO: 213 - protein, 9 aa, synthetic construct
  REGION 1..9: note = peptide
SDIAIDDVK

SEQ ID NO: 214 - protein, 8 aa, synthetic construct
  REGION 1..8: note = peptide
LGAETLPR

SEQ ID NO: 215 - protein, 10 aa, synthetic construct
  REGION 1..10: note = peptide
TEAESWYQTK

SEQ ID NO: 216 - protein, 13 aa, synthetic construct
  REGION 1..13: note = peptide
LVEIVHPSQEEDR

SEQ ID NO: 217 - protein, 8 aa, synthetic construct
  REGION 1..8: note = peptide
GSYYDSFK

SEQ ID NO: 218 - protein, 10 aa, synthetic construct
  REGION 1..10: note = peptide
GTYSTTVTGR

SEQ ID NO: 219 - protein, 7 aa, synthetic construct
  REGION 1..7: note = peptide
IVLVDNK

SEQ ID NO: 220 - protein, 9 aa, synthetic construct
  REGION 1..9: note = peptide
NPSDEDLLR

SEQ ID NO: 221 - protein, 11 aa, synthetic construct
  REGION 1..11: note = peptide
ETLDAQTFHTR

SEQ ID NO: 222 - protein, 8 aa, synthetic construct
  REGION 1..8: note = peptide
QLVEALDK

SEQ ID NO: 223 - protein, 12 aa, synthetic construct
  REGION 1..12: note = peptide
GEAAGAVQELAR

SEQ ID NO: 224 - protein, 12 aa, synthetic construct
  REGION 1..12: note = peptide
NFGGGNTAWEEK

SEQ ID NO: 225 - protein, 7 aa, synthetic construct
  REGION 1..7: note = peptide
GPLQLER

SEQ ID NO: 226 - protein, 7 aa, synthetic construct
  REGION 1..7: note = peptide
EDLTPFK

SEQ ID NO: 227 - protein, 9 aa, synthetic construct
  REGION 1..9: note = peptide
IQQNLDQLR

SEQ ID NO: 228 - protein, 7 aa, synthetic construct
  REGION 1..7: note = peptide
EALFGAR

SEQ ID NO: 229 - protein, 10 aa, synthetic construct
  REGION 1..10: note = peptide
YTSGFDELQR

SEQ ID NO: 230 - protein, 6 aa, synthetic construct
  REGION 1..6: note = peptide
LLQEIK

SEQ ID NO: 231 - protein, 8 aa, synthetic construct
  REGION 1..8: note = peptide
DLETSLEK

SEQ ID NO: 232 - protein, 7 aa, synthetic construct
  REGION 1..7: note = peptide
YLQSLER

SEQ ID NO: 233 - protein, 8 aa, synthetic construct
  REGION 1..8: note = peptide
FDPSLTQR

SEQ ID NO: 234 - protein, 11 aa, synthetic construct
  REGION 1..11: note = peptide
TYSVEYLDSSK

SEQ ID NO: 235 - protein, 10 aa, synthetic construct
  REGION 1..10: note = peptide
AGFAGDDAPR

SEQ ID NO: 236 - protein, 7 aa, synthetic construct
  REGION 1..7: note = peptide
TLTIQVK

SEQ ID NO: 237 - protein, 11 aa, synthetic construct
  REGION 1..11: note = peptide
SALTIQTLHTR

SEQ ID NO: 238 - protein, 8 aa, synthetic construct
  REGION 1..8: note = peptide
SYLPQTVR

SEQ ID NO: 239 - protein, 9 aa, synthetic construct
  REGION 1..9: note = peptide
YIFTATPAK

SEQ ID NO: 240 - protein, 10 aa, synthetic construct
  REGION 1..10: note = peptide
VTGVITQGAK

SEQ ID NO: 241 - protein, 10 aa, synthetic construct
  REGION 1..10: note = peptide
LPTDSELAPR

SEQ ID NO: 242 - protein, 8 aa, synthetic construct
  REGION 1..8: note = peptide
STDFFQSR

SEQ ID NO: 243 - protein, 9 aa, synthetic construct
  REGION 1..9: note = peptide
SLYNLGGSR

SEQ ID NO: 244 - protein, 11 aa, synthetic construct
  REGION 1..11: note = peptide
DTDLDGFPDEK

SEQ ID NO: 245 - protein, 8 aa, synthetic construct
  REGION 1..8: note = peptide
TFPISGAR

SEQ ID NO: 246 - protein, 6 aa, synthetic construct
  REGION 1..6: note = peptide
YLLEAK

SEQ ID NO: 247 - protein, 6 aa, synthetic construct
  REGION 1..6: note = peptide
ELLDYK

SEQ ID NO: 248 - protein, 7 aa, synthetic construct
  REGION 1..7: note = peptide
IDGVLIR

SEQ ID NO: 249 - protein, 9 aa, synthetic construct
  REGION 1..9: note = peptide
DISEVVTPR

SEQ ID NO: 250 - protein, 8 aa, synthetic construct
  REGION 1..8: note = peptide
TTGSGLLK

SEQ ID NO: 251 - protein, 8 aa, synthetic construct
  REGION 1..8: note = peptide
FDQNLDTK

SEQ ID NO: 252 - protein, 8 aa, synthetic construct
  REGION 1..8: note = peptide
LWEGSTSR

SEQ ID NO: 253 - protein, 12 aa, synthetic construct
  REGION 1..12: note = peptide
TNQVNSGGVLLR

SEQ ID NO: 254 - protein, 9 aa, synthetic construct
  REGION 1..9: note = peptide
LEGEPVALR

SEQ ID NO: 255 - protein, 9 aa, synthetic construct
  REGION 1..9: note = peptide
SAFSVAVTK

SEQ ID NO: 256 - protein, 9 aa, synthetic construct
  REGION 1..9: note = peptide
VDGSVDFYR

SEQ ID NO: 257 - protein, 9 aa, synthetic construct
  REGION 1..9: note = peptide
ETAALNSVR

SEQ ID NO: 258 - protein, 9 aa, synthetic construct
  REGION 1..9: note = peptide
ESGAEVYFR

SEQ ID NO: 259 - protein, 9 aa, synthetic construct
  REGION 1..9: note = peptide
FNDTEVLQR

SEQ ID NO: 260 - protein, 14 aa, synthetic construct
  REGION 1..14: note = peptide
IQALQQQADEAEDR

SEQ ID NO: 261 - protein, 7 aa, synthetic construct
  REGION 1..7: note = peptide
SLFTEGR

SEQ ID NO: 262 - protein, 7 aa, synthetic construct
  REGION 1..7: note = peptide
AYPTPLR

SEQ ID NO: 263 - protein, 8 aa, synthetic construct
  REGION 1..8: note = peptide
ATVFLEQR

SEQ ID NO: 264 - protein, 10 aa, synthetic construct
  REGION 1..10: note = peptide
EVGQLAETQR

SEQ ID NO: 265 - protein, 9 aa, synthetic construct
  REGION 1..9: note = peptide
LPVSLSSAK

SEQ ID NO: 266 - protein, 11 aa, synthetic construct
  REGION 1..11: note = peptide
QLYGDTGVLGR

SEQ ID NO: 267 - protein, 8 aa, synthetic construct
  REGION 1..8: note = peptide
AEIEYLEK

SEQ ID NO: 268 - protein, 9 aa, synthetic construct
  REGION 1..9: note = peptide
AAYLSTISK

SEQ ID NO: 269 - protein, 8 aa, synthetic construct
  REGION 1..8: note = peptide
LTQLNLDR

SEQ ID NO: 270 - protein, 9 aa, synthetic construct
  REGION 1..9: note = peptide
GQTLLAVAK

SEQ ID NO: 271 - protein, 7 aa, synthetic construct
  REGION 1..7: note = peptide
VLSFSSR

SEQ ID NO: 272 - protein, 7 aa, synthetic construct
  REGION 1..7: note = peptide
SLGFVSK

SEQ ID NO: 273 - protein, 8 aa, synthetic construct
  REGION 1..8: note = peptide
VAQVSITK

SEQ ID NO: 274 - protein, 9 aa, synthetic construct
  REGION 1..9: note = peptide
GDSVVYGLR

SEQ ID NO: 275 - protein, 10 aa, synthetic construct
  REGION 1..10: note = peptide
YLQGSSVQLR

SEQ ID NO: 276 - protein, 7 aa, synthetic construct
  REGION 1..7: note = peptide
DYWSTVK

SEQ ID NO: 277 - protein, 11 aa, synthetic construct
  REGION 1..11: note = peptide
SESETYTLSSK

SEQ ID NO: 278 - protein, 8 aa, synthetic construct
  REGION 1..8: note = peptide
ESLAAELR

SEQ ID NO: 279 - protein, 11 aa, synthetic construct
  REGION 1..11: note = peptide
SNFQQPYITNR

SEQ ID NO: 280 - protein, 7 aa, synthetic construct
  REGION 1..7: note = peptide
VLQGLPR

SEQ ID NO: 281 - protein, 8 aa, synthetic construct
  REGION 1..8: note = peptide
NWQDYGVR

SEQ ID NO: 282 - protein, 5 aa, synthetic construct
  REGION 1..5: note = peptide
DLFDR

SEQ ID NO: 283 - protein, 8 aa, synthetic construct
  REGION 1..8: note = peptide
ELVYETVR

SEQ ID NO: 284 - protein, 8 aa, synthetic construct
  REGION 1..8: note = peptide
SELVVEVK

SEQ ID NO: 285 - protein, 6 aa, synthetic construct
  REGION 1..6: note = peptide
YFQGIR

SEQ ID NO: 286 - protein, 8 aa, synthetic construct
  REGION 1..8: note = peptide
QINDYVAK

SEQ ID NO: 287 - protein, 13 aa, synthetic construct
  REGION 1..13: note = peptide
GNPESSFNDENLR

SEQ ID NO: 288 - protein, 10 aa, synthetic construct
  REGION 1..10: note = peptide
GYFGDEQQIR

SEQ ID NO: 289 - protein, 8 aa, synthetic construct
  REGION 1..8: note = peptide
VEDIPLAR

SEQ ID NO: 290 - protein, 8 aa, synthetic construct
  REGION 1..8: note = peptide
NDLISATK

SEQ ID NO: 291 - protein, 8 aa, synthetic construct
  REGION 1..8: note = peptide
QINDYVEK

SEQ ID NO: 292 - protein, 12 aa, synthetic construct
  REGION 1..12: note = peptide
EDTPNSVWEPAK

SEQ ID NO: 293 - protein, 7 aa, synthetic construct
  REGION 1..7: note = peptide
LPPLPPR

SEQ ID NO: 294 - protein, 11 aa, synthetic construct
  REGION 1..11: note = peptide
FVSTTYSGVTR

SEQ ID NO: 295 - protein, 8 aa, synthetic construct
  REGION 1..8: note = peptide
DISLSDYK

SEQ ID NO: 296 - protein, 11 aa, synthetic construct
  REGION 1..11: note = peptide
AAGASVVTELR

SEQ ID NO: 297 - protein, 11 aa, synthetic construct
  REGION 1..11: note = peptide
TFTPQPPGLER

SEQ ID NO: 298 - protein, 8 aa, synthetic construct
  REGION 1..8: note = peptide
IPALDPEK

SEQ ID NO: 299 - protein, 13 aa, synthetic construct
  REGION 1..13: note = peptide
VSSASDYNSSELK

SEQ ID NO: 300 - protein, 8 aa, synthetic construct
  REGION 1..8: note = peptide
YETELNLR

SEQ ID NO: 301 - protein, 11 aa, synthetic construct
  REGION 1..11: note = peptide
LVVVGAGGVGK

SEQ ID NO: 302 - protein, 5 aa, synthetic construct
  REGION 1..5: note = peptide
DFIYR

SEQ ID NO: 303 - protein, 8 aa, synthetic construct
  REGION 1..8: note = peptide
YLGEEYVK

SEQ ID NO: 304 - protein, 7 aa, synthetic construct
  REGION 1..7: note = peptide
LYTLVQR

SEQ ID NO: 305 - protein, 9 aa, synthetic construct
  REGION 1..9: note = peptide
GQVVYVFSK

SEQ ID NO: 306 - protein, 9 aa, synthetic construct
  REGION 1..9: note = peptide
LDVDQALNR

SEQ ID NO: 307 - protein, 8 aa, synthetic construct
  REGION 1..8: note = peptide
LESLLEEK

SEQ ID NO: 308 - protein, 9 aa, synthetic construct
  REGION 1..9: note = peptide
IIEGEPNLK

SEQ ID NO: 309 - protein, 10 aa, synthetic construct
  REGION 1..10: note = peptide
GVTSFGLENK

SEQ ID NO: 310 - protein, 11 aa, synthetic construct
  REGION 1..11: note = peptide
LTISESSISDR

SEQ ID NO: 311 - protein, 10 aa, synthetic construct
  REGION 1..10: note = peptide
VGDYGSLSGR

SEQ ID NO: 312 - protein, 10 aa, synthetic construct
  REGION 1..10: note = peptide
EPNAQEILQR

SEQ ID NO: 313 - protein, 8 aa, synthetic construct
  REGION 1..8: note = peptide
SFLDSGYR

SEQ ID NO: 314 - protein, 17 aa, synthetic construct
  REGION 1..17: note = peptide
SFHHEESLEELPETSGK

SEQ ID NO: 315 - protein, 11 aa, synthetic construct
  REGION 1..11: note = peptide
DQYYNIDVPSR

SEQ ID NO: 316 - protein, 7 aa, synthetic construct
  REGION 1..7: note = peptide
NIDVLEK

SEQ ID NO: 317 - protein, 9 aa, synthetic construct
  REGION 1..9: note = peptide
DLVQPINPR

SEQ ID NO: 318 - protein, 8 aa, synthetic construct
  REGION 1..8: note = peptide
INPASLDK

SEQ ID NO: 319 - protein, 8 aa, synthetic construct
  REGION 1..8: note = peptide
ADVNVLTK

SEQ ID NO: 320 - protein, 11 aa, synthetic construct
  REGION 1..11: note = peptide
AAGAPLATELR

SEQ ID NO: 321 - protein, 7 aa, synthetic construct
  REGION 1..7: note = peptide
QSIVPLR

SEQ ID NO: 322 - protein, 14 aa, synthetic construct
  REGION 1..14: note = peptide
GGSPPAPLPAHLSR

SEQ ID NO: 323 - protein, 9 aa, synthetic construct
  REGION 1..9: note = peptide
TEFTTALQR

SEQ ID NO: 324 - protein, 8 aa, synthetic construct
  REGION 1..8: note = peptide
SYVITTSR

SEQ ID NO: 325 - protein, 11 aa, synthetic construct
  REGION 1..11: note = peptide
DAVEDLESVGK

SEQ ID NO: 326 - protein, 6 aa, synthetic construct
  REGION 1..6: note = peptide
FLLYNR

SEQ ID NO: 327 - protein, 10 aa, synthetic construct
  REGION 1..10: note = peptide
QVIDVLETDK

SEQ ID NO: 328 - protein, 8 aa, synthetic construct
  REGION 1..8: note = peptide
TEEFEVTK

SEQ ID NO: 329 - protein, 10 aa, synthetic construct
  REGION 1..10: note = peptide
GLQAQGYGVR

SEQ ID NO: 330 - protein, 8 aa, synthetic construct
  REGION 1..8: note = peptide
ITDFGLAK

SEQ ID NO: 331 - protein, 9 aa, synthetic construct
  REGION 1..9: note = peptide
LEPESEFYR

SEQ ID NO: 332 - protein, 8 aa, synthetic construct
  REGION 1..8: note = peptide
ANSFLGEK

SEQ ID NO: 333 - protein, 11 aa, synthetic construct
  REGION 1..11: note = peptide
GNQWVGYDDVK

SEQ ID NO: 334 - protein, 10 aa, synthetic construct
  REGION 1..10: note = peptide
DADPDTFFAK

SEQ ID NO: 335 - protein, 8 aa, synthetic construct
  REGION 1..8: note = peptide
VVTITLDK

SEQ ID NO: 336 - protein, 11 aa, synthetic construct
  REGION 1..11: note = peptide
DFYVDENTTVR

SEQ ID NO: 337 - protein, 8 aa, synthetic construct
  REGION 1..8: note = peptide
YLVAPDGK

SEQ ID NO: 338 - protein, 10 aa, synthetic construct
  REGION 1..10: note = peptide
GSPILLGVSK

SEQ ID NO: 339 - protein, 8 aa, synthetic construct
  REGION 1..8: note = peptide
DLGSELVR

SEQ ID NO: 340 - protein, 9 aa, synthetic construct
  REGION 1..9: note = peptide
FSISNANIK

SEQ ID NO: 341 - protein, 10 aa, synthetic construct
  REGION 1..10: note = peptide
GLLPTSVSPR

SEQ ID NO: 342 - protein, 12 aa, synthetic construct
  REGION 1..12: note = peptide
YGLHVSPAYEGR

SEQ ID NO: 343 - protein, 12 aa, synthetic construct
  REGION 1..12: note = peptide
GPGLNLTSGQYR

SEQ ID NO: 344 - protein, 5 aa, synthetic construct
  REGION 1..5: note = peptide
TFYLR

SEQ ID NO: 345 - protein, 11 aa, synthetic construct
  REGION 1..11: note = peptide
YPDTLLGSSEK

SEQ ID NO: 346 - protein, 10 aa, synthetic construct
  REGION 1..10: note = peptide
LSEEEFGGFR

SEQ ID NO: 347 - protein, 9 aa, synthetic construct
  REGION 1..9: note = peptide
QEYEQLIAK

SEQ ID NO: 348 - protein, 9 aa, synthetic construct
  REGION 1..9: note = peptide
SLHVPGLNK

SEQ ID NO: 349 - protein, 8 aa, synthetic construct
  REGION 1..8: note = peptide
TVIEVDER

SEQ ID NO: 350 - protein, 9 aa, synthetic construct
  REGION 1..9: note = peptide
SLETSAFVK

SEQ ID NO: 351 - protein, 13 aa, synthetic construct
  REGION 1..13: note = peptide
SDDEVDDPAVELK

SEQ ID NO: 352 - protein, 12 aa, synthetic construct
  REGION 1..12: note = peptide
AALPEGLPEASR

SEQ ID NO: 353 - protein, 10 aa, synthetic construct
  REGION 1..10: note = peptide
QLDVEAALTK

SEQ ID NO: 354 - protein, 8 aa, synthetic construct
  REGION 1..8: note = peptide
LDSSEFLK

SEQ ID NO: 355 - protein, 8 aa, synthetic construct
  REGION 1..8: note = peptide
AVYEAVLR

SEQ ID NO: 356 - protein, 8 aa, synthetic construct
  REGION 1..8: note = peptide
VPTPQAIR

SEQ ID NO: 357 - protein, 10 aa, synthetic construct
  REGION 1..10: note = peptide
GWDWTSGVNK

SEQ ID NO: 358 - protein, 9 aa, synthetic construct
  REGION 1..9: note = peptide
VTVNVLSPR

SEQ ID NO: 359 - protein, 8 aa, synthetic construct
  REGION 1..8: note = peptide
FETEQALR

SEQ ID NO: 360 - protein, 10 aa, synthetic construct
  REGION 1..10: note = peptide
GQDTSEELLR

SEQ ID NO: 361 - protein, 7 aa, synthetic construct
  REGION 1..7: note = peptide
LSFSYGR

SEQ ID NO: 362 - protein, 11 aa, synthetic construct
  REGION 1..11: note = peptide
EVSFYYSEENK

SEQ ID NO: 363 - protein, 8 aa, synthetic construct
  REGION 1..8: note = peptide
APEGFAVR

SEQ ID NO: 364 - protein, 7 aa, synthetic construct
  REGION 1..7: note = peptide
DYPFQGK

SEQ ID NO: 365 - protein, 10 aa, synthetic construct
  REGION 1..10: note = peptide
LDGPLPSGVR

SEQ ID NO: 366 - protein, 10 aa, synthetic construct
  REGION 1..10: note = peptide
FSTQEEIQAR

SEQ ID NO: 367 - protein, 11 aa, synthetic construct
  REGION 1..11: note = peptide
AYQGVAAPFPK

SEQ ID NO: 368 - protein, 13 aa, synthetic construct
  REGION 1..13: note = peptide
ISPVEESEDVSNK

SEQ ID NO: 369 - protein, 8 aa, synthetic construct
  REGION 1..8: note = peptide
YSITFTGK

SEQ ID NO: 370 - protein, 6 aa, synthetic construct
  REGION 1..6: note = peptide
YQTWIK

SEQ ID NO: 371 - protein, 9 aa, synthetic construct
  REGION 1..9: note = peptide
QESFFVDER

SEQ ID NO: 372 - protein, 10 aa, synthetic construct
  REGION 1..10: note = peptide
QQDGELVGYR

SEQ ID NO: 373 - protein, 8 aa, synthetic construct
  REGION 1..8: note = peptide
FNVSSVEK

SEQ ID NO: 374 - protein, 10 aa, synthetic construct
  REGION 1..10: note = peptide
TDPGVFIGVK

SEQ ID NO: 375 - protein, 11 aa, synthetic construct
  REGION 1..11: note = peptide
AAGASVATELR

SEQ ID NO: 376 - protein, 11 aa, synthetic construct
  REGION 1..11: note = peptide
GEPGEGAYVYR

SEQ ID NO: 377 - protein, 12 aa, synthetic construct
  REGION 1..12: note = peptide
EAVILYAQPSER

SEQ ID NO: 378 - protein, 10 aa, synthetic construct
  REGION 1..10: note = peptide
GAVYVYFGSK

SEQ ID NO: 379 - protein, 10 aa, synthetic construct
  REGION 1..10: note = peptide
YQYAIDEYYR

SEQ ID NO: 380 - protein, 8 aa, synthetic construct
  REGION 1..8: note = peptide
TELLPGDR

SEQ ID NO: 381 - protein, 8 aa, synthetic construct
  REGION 1..8: note = peptide
DALEESLK

SEQ ID NO: 382 - protein, 13 aa, synthetic construct
  REGION 1..13: note = peptide
TEGDGVYTLNNEK

SEQ ID NO: 383 - protein, 7 aa, synthetic construct
  REGION 1..7: note = peptide
AFLGLQK

SEQ ID NO: 384 - protein, 13 aa, synthetic construct
  REGION 1..13: note = peptide
SPEAAGVQDPSLR

SEQ ID NO: 385 - protein, 8 aa, synthetic construct
  REGION 1..8: note = peptide
GNFVSPVK

SEQ ID NO: 386 - protein, 10 aa, synthetic construct
  REGION 1..10: note = peptide
IQNILTEEPK

SEQ ID NO: 387 - protein, 7 aa, synthetic construct
  REGION 1..7: note = peptide
DSEYPFK

SEQ ID NO: 388 - protein, 9 aa, synthetic construct
  REGION 1..9: note = peptide
ENYLLPEAK

SEQ ID NO: 389 - protein, 11 aa, synthetic construct
  REGION 1..11: note = peptide
DEGSYSLEEPK

SEQ ID NO: 390 - protein, 10 aa, synthetic construct
  REGION 1..10: note = peptide
VAQGIVSYGR

SEQ ID NO: 391 - protein, 8 aa, synthetic construct
  REGION 1..8: note = peptide
EQDQVWVR

SEQ ID NO: 392 - protein, 8 aa, synthetic construct
  REGION 1..8: note = peptide
SVPLPTLK

SEQ ID NO: 393 - protein, 12 aa, synthetic construct
  REGION 1..12: note = peptide
GNETLHYETFGK

SEQ ID NO: 394 - protein, 13 aa, synthetic construct
  REGION 1..13: note = peptide
NTQIDNSWGSEER

SEQ ID NO: 395 - protein, 8 aa, synthetic construct
  REGION 1..8: note = peptide
LLELTGPK

SEQ ID NO: 396 - protein, 10 aa, synthetic construct
  REGION 1..10: note = peptide
IQELQLAASR

SEQ ID NO: 397 - protein, 13 aa, synthetic construct
  REGION 1..13: note = peptide
LAAADGAVAGEVR

SEQ ID NO: 398 - protein, 9 aa, synthetic construct
  REGION 1..9: note = peptide
TAVNALWGK

SEQ ID NO: 399 - protein, 15 aa, synthetic construct
  REGION 1..15: note = peptide
VGAHAGEYGAEALER

SEQ ID NO: 400 - protein, 8 aa, synthetic construct
  REGION 1..8: note = peptide
LPGGLEPK

SEQ ID NO: 401 - protein, 6 aa, synthetic construct
  REGION 1..6: note = peptide
LAILYR

SEQ ID NO: 402 - protein, 13 aa, synthetic construct
  REGION 1..13: note = peptide
LPGGYGLPYTTGK

SEQ ID NO: 403 - protein, 9 aa, synthetic construct
  REGION 1..9: note = peptide
QLAEEYLYR

SEQ ID NO: 404 - protein, 11 aa, synthetic construct
  REGION 1..11: note = peptide
DITSDTSGDFR

SEQ ID NO: 405 - protein, 10 aa, synthetic construct
  REGION 1..10: note = peptide
AGGSIPIPQK

SEQ ID NO: 406 - protein, 7 aa, synthetic construct
  REGION 1..7: note = peptide
QNSLLWR

SEQ ID NO: 407 - protein, 8 aa, synthetic construct
  REGION 1..8: note = peptide
LPASFDAR

SEQ ID NO: 408 - protein, 9 aa, synthetic construct
  REGION 1..9: note = peptide
QIGEFIVTR

SEQ ID NO: 409 - protein, 8 aa, synthetic construct
  REGION 1..8: note = peptide
VIDEEWQR

SEQ ID NO: 410 - protein, 10 aa, synthetic construct
  REGION 1..10: note = peptide
ESDTSYVSLK

SEQ ID NO: 411 - protein, 10 aa, synthetic construct
  REGION 1..10: note = peptide
SDALQLGLGK

SEQ ID NO: 412 - protein, 10 aa, synthetic construct
  REGION 1..10: note = peptide
DVAVIAESIR

SEQ ID NO: 413 - protein, 11 aa, synthetic construct
  REGION 1..11: note = peptide
DSLSINATNIK

SEQ ID NO: 414 - protein, 8 aa, synthetic construct
  REGION 1..8: note = peptide
LAYYGFTK

SEQ ID NO: 415 - protein, 7 aa, synthetic construct
  REGION 1..7: note = peptide
GVQINIK

SEQ ID NO: 416 - protein, 9 aa, synthetic construct
  REGION 1..9: note = peptide
ALLAFQESK

SEQ ID NO: 417 - protein, 11 aa, synthetic construct
  REGION 1..11: note = peptide
SVIAPSLEQYK

SEQ ID NO: 418 - protein, 17 aa, synthetic construct
  REGION 1..17: note = peptide
GTHSLPPRPAAVPVPLR

SEQ ID NO: 419 - protein, 10 aa, synthetic construct
  REGION 1..10: note = peptide
YEELQVTVGR

SEQ ID NO: 420 - protein, 15 aa, synthetic construct
  REGION 1..15: note = peptide
SQASPSEDEETFELR

SEQ ID NO: 421 - protein, 8 aa, synthetic construct
  REGION 1..8: note = peptide
YTELPYGR

SEQ ID NO: 422 - protein, 8 aa, synthetic construct
  REGION 1..8: note = peptide
DFIDIESK

SEQ ID NO: 423 - protein, 8 aa, synthetic construct
  REGION 1..8: note = peptide
LTPEELER

SEQ ID NO: 424 - protein, 7 aa, synthetic construct
  REGION 1..7: note = peptide
VTWQNLR

SEQ ID NO: 425 - protein, 9 aa, synthetic construct
  REGION 1..9: note = peptide
VLDELTLSK

SEQ ID NO: 426 - protein, 8 aa, synthetic construct
  REGION 1..8: note = peptide
GIDPDLLK

SEQ ID NO: 427 - protein, 6 aa, synthetic construct
  REGION 1..6: note = peptide
AFVFPK

SEQ ID NO: 428 - protein, 9 aa, synthetic construct
  REGION 1..9: note = peptide
TAAIVNSIR

SEQ ID NO: 429 - protein, 13 aa, synthetic construct
  REGION 1..13: note = peptide
NGSQAFVHWQEPR

SEQ ID NO: 430 - protein, 9 aa, synthetic construct
  REGION 1..9: note = peptide
ELLETVVNR

SEQ ID NO: 431 - protein, 8 aa, synthetic construct
  REGION 1..8: note = peptide
DLNETLLR

SEQ ID NO: 432 - protein, 9 aa, synthetic construct
  REGION 1..9: note = peptide
QDGSVDFFR

SEQ ID NO: 433 - protein, 11 aa, synthetic construct
  REGION 1..11: note = peptide
TSNFNAAISLK

SEQ ID NO: 434 - protein, 9 aa, synthetic construct
  REGION 1..9: note = peptide
EATLELLGR

SEQ ID NO: 435 - protein, 8 aa, synthetic construct
  REGION 1..8: note = peptide
AEIYALNR

SEQ ID NO: 436 - protein, 8 aa, synthetic construct
  REGION 1..8: note = peptide
ALLEAPLK

SEQ ID NO: 437 - protein, 8 aa, synthetic construct
  REGION 1..8: note = peptide
IELPTTVK

SEQ ID NO: 438 - protein, 8 aa, synthetic construct
  REGION 1..8: note = peptide
VLFSGSLR

SEQ ID NO: 439 - protein, 8 aa, synthetic construct
  REGION 1..8: note = peptide
EVEQVYLR

SEQ ID NO: 440 - protein, 14 aa, synthetic construct
  REGION 1..14: note = peptide
LPGIFDDVHGSHGR

SEQ ID NO: 441 - protein, 11 aa, synthetic construct
  REGION 1..11: note = peptide
GTPLPTYEEAK

SEQ ID NO: 442 - protein, 9 aa, synthetic construct
  REGION 1..9: note = peptide
TVPDPLAVK

SEQ ID NO: 443 - protein, 8 aa, synthetic construct
  REGION 1..8: note = peptide
LQQQLWSK

SEQ ID NO: 444 - protein, 11 aa, synthetic construct
  REGION 1..11: note = peptide
SQLEESISQLR

SEQ ID NO: 445 - protein, 8 aa, synthetic construct
  REGION 1..8: note = peptide
QELTTEFR

SEQ ID NO: 446 - protein, 6 aa, synthetic construct
  REGION 1..6: note = peptide
LYDVLR

SEQ ID NO: 447 - protein, 9 aa, synthetic construct
  REGION 1..9: note = peptide
TVLFGVQPK

SEQ ID NO: 448 - protein, 12 aa, synthetic construct
  REGION 1..12: note = peptide
LSVVGYSGSAGR

SEQ ID NO: 449 - protein, 9 aa, synthetic construct
  REGION 1..9: note = peptide
LFAYPDTHR

SEQ ID NO: 450 - protein, 11 aa, synthetic construct
  REGION 1..11: note = peptide
ISISTSGGSFR

SEQ ID NO: 451 - protein, 10 aa, synthetic construct
  REGION 1..10: note = peptide
LSPEYYDLAR

SEQ ID NO: 452 - protein, 12 aa, synthetic construct
  REGION 1..12: note = peptide
ALPSHLGLHPER

SEQ ID NO: 453 - protein, 8 aa, synthetic construct
  REGION 1..8: note = peptide
YEVVYPIR

SEQ ID NO: 454 - protein, 7 aa, synthetic construct
  REGION 1..7: note = peptide
ALFSTLK

SEQ ID NO: 455 - protein, 6 aa, synthetic construct
  REGION 1..6: note = peptide
IQILPR

SEQ ID NO: 456 - protein, 10 aa, synthetic construct
  REGION 1..10: note = peptide
SGPTWWGPQR

SEQ ID NO: 457 - protein, 11 aa, synthetic construct
  REGION 1..11: note = peptide
GLQVALEEFHK

SEQ ID NO: 458 - protein, 10 aa, synthetic construct
  REGION 1..10: note = peptide
LGDGFEGFYK

SEQ ID NO: 459 - protein, 9 aa, synthetic construct
  REGION 1..9: note = peptide
VVGGLVALR

SEQ ID NO: 460 - protein, 8 aa, synthetic construct
  REGION 1..8: note = peptide
VSPLTFGR

SEQ ID NO: 461 - protein, 12 aa, synthetic construct
  REGION 1..12: note = peptide
TATITVLPQQPR

SEQ ID NO: 462 - protein, 11 aa, synthetic construct
  REGION 1..11: note = peptide
SANTITSFVDR

SEQ ID NO: 463 - protein, 10 aa, synthetic construct
  REGION 1..10: note = peptide
NSWGENWGNK

SEQ ID NO: 464 - protein, 10 aa, synthetic construct
  REGION 1..10: note = peptide
VGDQPTLQLK

SEQ ID NO: 465 - protein, 12 aa, synthetic construct
  REGION 1..12: note = peptide
ELLEEVGQNGSR

SEQ ID NO: 466 - protein, 10 aa, synthetic construct
  REGION 1..10: note = peptide
NVIDPPIYAR

SEQ ID NO: 467 - protein, 9 aa, synthetic construct
  REGION 1..9: note = peptide
VLFYVDSEK

SEQ ID NO: 468 - protein, 10 aa, synthetic construct
  REGION 1..10: note = peptide
GSEIVAGLEK

SEQ ID NO: 469 - protein, 9 aa, synthetic construct
  REGION 1..9: note = peptide
GLVVLTPER

SEQ ID NO: 470 - protein, 10 aa, synthetic construct
  REGION 1..10: note = peptide
AVPEGFVIPR

SEQ ID NO: 471 - protein, 12 aa, synthetic construct
  REGION 1..12: note = peptide
GWSTDEANTYFK

SEQ ID NO: 472 - protein, 11 aa, synthetic construct
  REGION 1..11: note = peptide
GVAETPTYPWR

SEQ ID NO: 473 - protein, 13 aa, synthetic construct
  REGION 1..13: note = peptide
WSGDFTQGPQSAK

SEQ ID NO: 474 - protein, 10 aa, synthetic construct
  REGION 1..10: note = peptide
LLLGTGTDAR

SEQ ID NO: 475 - protein, 9 aa, synthetic construct
  REGION 1..9: note = peptide
GLSGIGAFR

SEQ ID NO: 476 - protein, 14 aa, synthetic construct
  REGION 1..14: note = peptide
ESESAPGDFSLSVK

SEQ ID NO: 477 - protein, 8 aa, synthetic construct
  REGION 1..8: note = peptide
DFIATLGK

SEQ ID NO: 478 - protein, 14 aa, synthetic construct
  REGION 1..14: note = peptide
SFISGGSTITGVGK

SEQ ID NO: 479 - protein, 13 aa, synthetic construct
  REGION 1..13: note = peptide
GVSPSASAWPEEK

SEQ ID NO: 480 - protein, 11 aa, synthetic construct
  REGION 1..11: note = peptide
DTNALPPTVFK

SEQ ID NO: 481 - protein, 8 aa, synthetic construct
  REGION 1..8: note = peptide
IFGSYDPR

SEQ ID NO: 482 - protein, 7 aa, synthetic construct
  REGION 1..7: note = peptide
SLTEILK

SEQ ID NO: 483 - protein, 12 aa, synthetic construct
  REGION 1..12: note = peptide
TLEPELGTLQAR

SEQ ID NO: 484 - protein, 12 aa, synthetic construct
  REGION 1..12: note = peptide
SGLSTGWTQLSK

SEQ ID NO: 485 - protein, 11 aa, synthetic construct
  REGION 1..11: note = peptide
EEADALYEALK

SEQ ID NO: 486 - protein, 9 aa, synthetic construct
  REGION 1..9: note = peptide
IAQYYYTFK

SEQ ID NO: 487 - protein, 8 aa, synthetic construct
  REGION 1..8: note = peptide
IEVAQFVK

SEQ ID NO: 488 - protein, 11 aa, synthetic construct
  REGION 1..11: note = peptide
AELAETIVYAR

SEQ ID NO: 489 - protein, 8 aa, synthetic construct
  REGION 1..8: note = peptide
FFQYDTWK

SEQ ID NO: 490 - protein, 11 aa, synthetic construct
  REGION 1..11: note = peptide
LYTDDEDDIYK

SEQ ID NO: 491 - protein, 12 aa, synthetic construct
  REGION 1..12: note = peptide
DNIYTSEVVSQR

SEQ ID NO: 492 - protein, 8 aa, synthetic construct
  REGION 1..8: note = peptide
QLVLNVSK

SEQ ID NO: 493 - protein, 11 aa, synthetic construct
  REGION 1..11: note = peptide
ALDFAVGEYNK

SEQ ID NO: 494 - protein, 9 aa, synthetic construct
  REGION 1..9: note = peptide
YLGVTLSPR

SEQ ID NO: 495 - protein, 9 aa, synthetic construct
  REGION 1..9: note = peptide
TTTLPVEFK

SEQ ID NO: 496 - protein, 9 aa, synthetic construct
  REGION 1..9: note = peptide
TGIIDYGIR

SEQ ID NO: 497 - protein, 12 aa, synthetic construct
  REGION 1..12: note = peptide
EQPELEVQYQGR

SEQ ID NO: 498 - protein, 9 aa, synthetic construct
  REGION 1..9: note = peptide
SWSVYVGAR

SEQ ID NO: 499 - protein, 7 aa, synthetic construct
  REGION 1..7: note = peptide
WVQDYIK

SEQ ID NO: 500 - protein, 14 aa, synthetic construct
  REGION 1..14: note = peptide
GDLTIANLGTSEGR

SEQ ID NO: 501 - protein, 8 aa, synthetic construct
  REGION 1..8: note = peptide
DALSALAR

SEQ ID NO: 502 - protein, 7 aa, synthetic construct
  REGION 1..7: note = peptide
LALFPDK

SEQ ID NO: 503 - protein, 10 aa, synthetic construct
  REGION 1..10: note = peptide
SGLNIEDLEK

SEQ ID NO: 504 - protein, 13 aa, synthetic construct
  REGION 1..13: note = peptide
AQATPWTQTQAVR

SEQ ID NO: 505 - protein, 11 aa, synthetic construct
  REGION 1..11: note = peptide
SLDSPAALAER

SEQ ID NO: 506 - protein, 9 aa, synthetic construct
  REGION 1..9: note = peptide
YGGDPPWPR

SEQ ID NO: 507 - protein, 8 aa, synthetic construct
  REGION 1..8: note = peptide
QWAGLVEK

SEQ ID NO: 508 - protein, 12 aa, synthetic construct
  REGION 1..12: note = peptide
TSFPEDTVITYK

SEQ ID NO: 509 - protein, 9 aa, synthetic construct
  REGION 1..9: note = peptide
NYNLVESLK

SEQ ID NO: 510 - protein, 9 aa, synthetic construct
  REGION 1..9: note = peptide
LYIEYGIQR

SEQ ID NO: 511 - protein, 11 aa, synthetic construct
  REGION 1..11: note = peptide
VEPSVFLPASK

SEQ ID NO: 512 - protein, 11 aa, synthetic construct
  REGION 1..11: note = peptide
DGGVLSPILTR

SEQ ID NO: 513 - protein, 9 aa, synthetic construct
  REGION 1..9: note = peptide
VLDELTLTK

SEQ ID NO: 514 - protein, 11 aa, synthetic construct
  REGION 1..11: note = peptide
LDIGIINENQR

SEQ ID NO: 515 - protein, 11 aa, synthetic construct
  REGION 1..11: note = peptide
LPEPIVSTDSR

SEQ ID NO: 516 - protein, 10 aa, synthetic construct
  REGION 1..10: note = peptide
EENDDFASFR

SEQ ID NO: 517 - protein, 9 aa, synthetic construct
  REGION 1..9: note = peptide
TILFSYGTK

SEQ ID NO: 518 - protein, 8 aa, synthetic construct
  REGION 1..8: note = peptide
SQFEGFVK

SEQ ID NO: 519 - protein, 6 aa, synthetic construct
  REGION 1..6: note = peptide
LDPFFK

SEQ ID NO: 520 - protein, 11 aa, synthetic construct
  REGION 1..11: note = peptide
DSDLLSPSDFK

SEQ ID NO: 521 - protein, 9 aa, synthetic construct
  REGION 1..9: note = peptide
ALENLLPTK

SEQ ID NO: 522 - protein, 11 aa, synthetic construct
  REGION 1..11: note = peptide
TIELLGQEVSR

SEQ ID NO: 523 - protein, 13 aa, synthetic construct
  REGION 1..13: note = peptide
VGYPGPSGPLGAR

SEQ ID NO: 524 - protein, 11 aa, synthetic construct
  REGION 1..11: note = peptide
NFPSPVDAAFR

SEQ ID NO: 525 - protein, 6 aa, synthetic construct
  REGION 1..6: note = peptide
YISLLK

SEQ ID NO: 526 - protein, 13 aa, synthetic construct
  REGION 1..13: note = peptide
IPQEEFDGNQFQK

SEQ ID NO: 527 - protein, 9 aa, synthetic construct
  REGION 1..9: note = peptide
SAVTALWGK

SEQ ID NO: 528 - protein, 11 aa, synthetic construct
  REGION 1..11: note = peptide
LSILYPATTGR

SEQ ID NO: 529 - protein, 8 aa, synthetic construct
  REGION 1..8: note = peptide
LFLETAEK

SEQ ID NO: 530 - protein, 8 aa, synthetic construct
  REGION 1..8: note = peptide
QLEWGLER

SEQ ID NO: 531 - protein, 8 aa, synthetic construct
  REGION 1..8: note = peptide
IIVPLNNR

SEQ ID NO: 532 - protein, 8 aa, synthetic construct
  REGION 1..8: note = peptide
DDFLIYDR

SEQ ID NO: 533 - protein, 9 aa, synthetic construct
  REGION 1..9: note = peptide
AGYYYIYSK

SEQ ID NO: 534 - protein, 12 aa, synthetic construct
  REGION 1..12: note = peptide
TPASQGVILPIK

SEQ ID NO: 535 - protein, 7 aa, synthetic construct
  REGION 1..7: note = peptide
NTVLVWR

SEQ ID NO: 536 - protein, 10 aa, synthetic construct
  REGION 1..10: note = peptide
IVEELQSLSK

SEQ ID NO: 537 - protein, 10 aa, synthetic construct
  REGION 1..10: note = peptide
TFYNASWSSR

SEQ ID NO: 538 - protein, 13 aa, synthetic construct
  REGION 1..13: note = peptide
QEVWLANGAAESR

SEQ ID NO: 539 - protein, 10 aa, synthetic construct
  REGION 1..10: note = peptide
ISVPYEGVFR

SEQ ID NO: 540 - protein, 12 aa, synthetic construct
  REGION 1..12: note = peptide
IIDGVPVEITEK

SEQ ID NO: 541 - protein, 11 aa, synthetic construct
  REGION 1..11: note = peptide
FQLFGSPSGQK

SEQ ID NO: 542 - protein, 9 aa, synthetic construct
  REGION 1..9: note = peptide
ANVFVQLPR

SEQ ID NO: 543 - protein, 11 aa, synthetic construct
  REGION 1..11: note = peptide
AQWANPFDPSK

SEQ ID NO: 544 - protein, 7 aa, synthetic construct
  REGION 1..7: note = peptide
LAAWLAK

SEQ ID NO: 545 - protein, 7 aa, synthetic construct
  REGION 1..7: note = peptide
YYTVFDR

SEQ ID NO: 546 - protein, 13 aa, synthetic construct
  REGION 1..13: note = peptide
EFSEENPAQNLPK

SEQ ID NO: 547 - protein, 8 aa, synthetic construct
  REGION 1..8: note = peptide
FTGSSWIK

SEQ ID NO: 548 - protein, 7 aa, synthetic construct
  REGION 1..7: note = peptide
IWLDNVR

SEQ ID NO: 549 - protein, 8 aa, synthetic construct
  REGION 1..8: note = peptide
ETLLQDFR

SEQ ID NO: 550 - protein, 10 aa, synthetic construct
  REGION 1..10: note = peptide
LTFYGNWSEK

SEQ ID NO: 551 - protein, 11 aa, synthetic construct
  REGION 1..11: note = peptide
QLVPALGPPVR

SEQ ID NO: 552 - protein, 9 aa, synthetic construct
  REGION 1..9: note = peptide
ENYPLPWEK

SEQ ID NO: 553 - protein, 10 aa, synthetic construct
  REGION 1..10: note = peptide
LELQQLQAER

SEQ ID NO: 554 - protein, 8 aa, synthetic construct
  REGION 1..8: note = peptide
IVIEYVDR

SEQ ID NO: 555 - protein, 9 aa, synthetic construct
  REGION 1..9: note = peptide
IPVDLPEAR

SEQ ID NO: 556 - protein, 12 aa, synthetic construct
  REGION 1..12: note = peptide
DPTFIPAPIQAK

SEQ ID NO: 557 - protein, 13 aa, synthetic construct
  REGION 1..13: note = peptide
QQPLFVSGGDDYK

SEQ ID NO: 558 - protein, 13 aa, synthetic construct
  REGION 1..13: note = peptide
VLLPPDYSEDGAR

SEQ ID NO: 559 - protein, 7 aa, synthetic construct
  REGION 1..7: note = peptide
FVSFLGR

SEQ ID NO: 560 - protein, 8 aa, synthetic construct
  REGION 1..8: note = peptide
FSAEFDFR

SEQ ID NO: 561 - protein, 9 aa, synthetic construct
  REGION 1..9: note = peptide
DQEAPYLLR

SEQ ID NO: 562 - protein, 7 aa, synthetic construct
  REGION 1..7: note = peptide
AFLLTPR

SEQ ID NO: 563 - protein, 8 aa, synthetic construct
  REGION 1..8: note = peptide
WAFNWDTK

SEQ ID NO: 564 - protein, 12 aa, synthetic construct
  REGION 1..12: note = peptide
STDYGIFQINSR

SEQ ID NO: 565 - protein, 12 aa, synthetic construct
  REGION 1..12: note = peptide
DSPSVWAAVPGK

SEQ ID NO: 566 - protein, 13 aa, synthetic construct
  REGION 1..13: note = peptide
VEYITGPGVTTYK

SEQ ID NO: 567 - protein, 8 aa, synthetic construct
  REGION 1..8: note = peptide
LLPYVLEK

SEQ ID NO: 568 - protein, 10 aa, synthetic construct
  REGION 1..10: note = peptide
LVIIEGDLER

SEQ ID NO: 569 - protein, 8 aa, synthetic construct
  REGION 1..8: note = peptide
TVIYEIPR

SEQ ID NO: 570 - protein, 10 aa, synthetic construct
  REGION 1..10: note = peptide
GPPAALTLPR

SEQ ID NO: 571 - protein, 8 aa, synthetic construct
  REGION 1..8: note = peptide
TPLYIDFK

SEQ ID NO: 572 - protein, 11 aa, synthetic construct
  REGION 1..11: note = peptide
NLQEILHGAVR

SEQ ID NO: 573 - protein, 13 aa, synthetic construct
  REGION 1..13: note = peptide
LLDLGAGDGEVTK

SEQ ID NO: 574 - protein, 10 aa, synthetic construct
  REGION 1..10: note = peptide
DTSLFSDEFK

SEQ ID NO: 575 - protein, 13 aa, synthetic construct
  REGION 1..13: note = peptide
YSSDYFQAPSDYR

SEQ ID NO: 576 - protein, 13 aa, synthetic construct
  REGION 1..13: note = peptide
IPEGEAVTAAEFR

SEQ ID NO: 577 - protein, 11 aa, synthetic construct
  REGION 1..11: note = peptide
EGYYGYTGAFR

SEQ ID NO: 578 - protein, 12 aa, synthetic construct
  REGION 1..12: note = peptide
EGHFYYNISEVK

SEQ ID NO: 579 - protein, 14 aa, synthetic construct
  REGION 1..14: note = peptide
DSTYSLSSTLTLSK

SEQ ID NO: 580 - protein, 12 aa, synthetic construct
  REGION 1..12: note = peptide
NGSGPFLGNIPK

SEQ ID NO: 581 - protein, 9 aa, synthetic construct
  REGION 1..9: note = peptide
YGNLSNFLR

SEQ ID NO: 582 - protein, 13 aa, synthetic construct
  REGION 1..13: note = peptide
GNPTVEVDLYTAK

SEQ ID NO: 583 - protein, 7 aa, synthetic construct
  REGION 1..7: note = peptide
VYLPWSR

SEQ ID NO: 584 - protein, 8 aa, synthetic construct
  REGION 1..8: note = peptide
YLPLENLR

SEQ ID NO: 585 - protein, 12 aa, synthetic construct
  REGION 1..12: note = peptide
VYSGILNQSEIK

SEQ ID NO: 586 - protein, 8 aa, synthetic construct
  REGION 1..8: note = peptide
FPLTNAIK

SEQ ID NO: 587 - protein, 15 aa, synthetic construct
  REGION 1..15: note = peptide
VIEASFPAGVDSSPR

SEQ ID NO: 588 - protein, 8 aa, synthetic construct
  REGION 1..8: note = peptide
TWYPEVPK

SEQ ID NO: 589 - protein, 12 aa, synthetic construct
  REGION 1..12: note = peptide
QIFLPEPEQPSR

SEQ ID NO: 590 - protein, 13 aa, synthetic construct
  REGION 1..13: note = peptide
QELIQAEIQNGVK

SEQ ID NO: 591 - protein, 11 aa, synthetic construct
  REGION 1..11: note = peptide
GDLYFANVEEK

SEQ ID NO: 592 - protein, 11 aa, synthetic construct
  REGION 1..11: note = peptide
GWVTDGFSSLK

SEQ ID NO: 593 - protein, 13 aa, synthetic construct
  REGION 1..13: note = peptide
VDAETGDVFAIER

SEQ ID NO: 594 - protein, 8 aa, synthetic construct
  REGION 1..8: note = peptide
LFQIQFNR

SEQ ID NO: 595 - protein, 13 aa, synthetic construct
  REGION 1..13: note = peptide
AQDGGPVGTELFR

SEQ ID NO: 596 - protein, 12 aa, synthetic construct
  REGION 1..12: note = peptide
YGSQLAPETFYR

SEQ ID NO: 597 - protein, 10 aa, synthetic construct
  REGION 1..10: note = peptide
LSSPAVITDK

SEQ ID NO: 598 - protein, 12 aa, synthetic construct
  REGION 1..12: note = peptide
AYSLFSYNTQGR

SEQ ID NO: 599 - protein, 13 aa, synthetic construct
  REGION 1..13: note = peptide
LAILGGVEGQPAK

SEQ ID NO: 600 - protein, 5 aa, synthetic construct
  REGION 1..5: note = peptide
DWFLR

SEQ ID NO: 601 - protein, 8 aa, synthetic construct
  REGION 1..8: note = peptide
YSFTIELR

SEQ ID NO: 602 - protein, 13 aa, synthetic construct
  REGION 1..13: note = peptide
AADDTWEPFASGK

SEQ ID NO: 603 - protein, 9 aa, synthetic construct
  REGION 1..9: note = peptide
LPGIFDDVR

SEQ ID NO: 604 - protein, 8 aa, synthetic construct
  REGION 1..8: note = peptide
ELTLEDLK

SEQ ID NO: 605 - protein, 12 aa, synthetic construct
  REGION 1..12: note = peptide
ESFEESWTPNYK

SEQ ID NO: 606 - protein, 9 aa, synthetic construct
  REGION 1..9: note = peptide
TSVPPFNLR

SEQ ID NO: 607 - protein, 11 aa, synthetic construct
  REGION 1..11: note = peptide
DYPDEVLQFAR

SEQ ID NO: 608 - protein, 8 aa, synthetic construct
  REGION 1..8: note = peptide
WIQEYLEK

SEQ ID NO: 609 - protein, 6 aa, synthetic construct
  REGION 1..6: note = peptide
FGIILR

SEQ ID NO: 610 - protein, 12 aa, synthetic construct
  REGION 1..12: note = peptide
FEDGVLDPDYPR

SEQ ID NO: 611 - protein, 9 aa, synthetic construct
  REGION 1..9: note = peptide
ANLTVVLLR

SEQ ID NO: 612 - protein, 12 aa, synthetic construct
  REGION 1..12: note = peptide
GSVQYLPDLDDK

SEQ ID NO: 613 - protein, 13 aa, synthetic construct
  REGION 1..13: note = peptide
LSDLEAQWAPSPR

SEQ ID NO: 614 - protein, 11 aa, synthetic construct
  REGION 1..11: note = peptide
LPLEYSYGEYR

SEQ ID NO: 615 - protein, 10 aa, synthetic construct
  REGION 1..10: note = peptide
FNAPFDVGIK

SEQ ID NO: 616 - protein, 17 aa, synthetic construct
  REGION 1..17: note = peptide
YLYTDDAQQTEAHLEIR

SEQ ID NO: 617 - protein, 6 aa, synthetic construct
  REGION 1..6: note = peptide
FYTFLK

SEQ ID NO: 618 - protein, 13 aa, synthetic construct
  REGION 1..13: note = peptide
VPPPSDAPLPFDR

SEQ ID NO: 619 - protein, 8 aa, synthetic construct
  REGION 1..8: note = peptide
FLNVLSPR

SEQ ID NO: 620 - protein, 8 aa, synthetic construct
  REGION 1..8: note = peptide
QFYSVFDR

SEQ ID NO: 621 - protein, 8 aa, synthetic construct
  REGION 1..8: note = peptide
TFTLLDPK

SEQ ID NO: 622 - protein, 13 aa, synthetic construct
  REGION 1..13: note = peptide
NSSAAWDETLLEK

SEQ ID NO: 623 - protein, 8 aa, synthetic construct
  REGION 1..8: note = peptide
LALAFYGR

SEQ ID NO: 624 - protein, 13 aa, synthetic construct
  REGION 1..13: note = peptide
DYVSQFEGSALGK

SEQ ID NO: 625 - protein, 13 aa, synthetic construct
  REGION 1..13: note = peptide
DSSAAWDEDLLDK

SEQ ID NO: 626 - protein, 8 aa, synthetic construct
  REGION 1..8: note = peptide
SWSWNYYR

SEQ ID NO: 627 - protein, 9 aa, synthetic construct
  REGION 1..9: note = peptide
ITFSPPLPR

SEQ ID NO: 628 - protein, 7 aa, synthetic construct
  REGION 1..7: note = peptide
VDLFYLR

SEQ ID NO: 629 - protein, 8 aa, synthetic construct
  REGION 1..8: note = peptide
LLWQLNGR

SEQ ID NO: 630 - protein, 13 aa, synthetic construct
  REGION 1..13: note = peptide
DSSATWEQSLLEK

SEQ ID NO: 631 - protein, 13 aa, synthetic construct
  REGION 1..13: note = peptide
NPLNAGSWEWSDR

SEQ ID NO: 632 - protein, 8 aa, synthetic construct
  REGION 1..8: note = peptide
YSVFPTLR

SEQ ID NO: 633 - protein, 13 aa, synthetic construct
  REGION 1..13: note = peptide
VTAGISFAIPSDK

SEQ ID NO: 634 - protein, 12 aa, synthetic construct
  REGION 1..12: note = peptide
FLASVSTVLTSK

SEQ ID NO: 635 - protein, 13 aa, synthetic construct
  REGION 1..13: note = peptide
QSWGLENEALIVR

SEQ ID NO: 636 - protein, 8 aa, synthetic construct
  REGION 1..8: note = peptide
FLVSLALR

SEQ ID NO: 637 - protein, 8 aa, synthetic construct
  REGION 1..8: note = peptide
EYFWGLSK

SEQ ID NO: 638 - protein, 13 aa, synthetic construct
  REGION 1..13: note = peptide
TVDNFVALATGEK

SEQ ID NO: 639 - protein, 10 aa, synthetic construct
  REGION 1..10: note = peptide
ALAAVLEELR

SEQ ID NO: 640 - protein, 12 aa, synthetic construct
  REGION 1..12: note = peptide
VGYPELAEVLGR

SEQ ID NO: 641 - protein, 8 aa, synthetic construct
  REGION 1..8: note = peptide
FTPWWETK

SEQ ID NO: 642 - protein, 9 aa, synthetic construct
  REGION 1..9: note = peptide
TLAFPLTIR

SEQ ID NO: 643 - protein, 13 aa, synthetic construct
  REGION 1..13: note = peptide
LPPWNPQVFSSER

SEQ ID NO: 644 - protein, 18 aa, synthetic construct
  REGION 1..18: note = peptide
SYELPDGQVITISNEWFR

SEQ ID NO: 645 - protein, 11 aa, synthetic construct
  REGION 1..11: note = peptide
WVAVVFPLSYR

SEQ ID NO: 646 - protein, 15 aa, synthetic construct
  REGION 1..15: note = peptide
TVAGQDAVIVLLGTR

SEQ ID NO: 647 - protein, 11 aa, synthetic construct
  REGION 1..11: note = peptide
VLLVELPAFLR

SEQ ID NO: 648 - protein, 4 aa, synthetic construct
  REGION 1..4: note = peptide
LVLK

SEQ ID NO: 649 - protein, 4 aa, synthetic construct
  REGION 1..4: note = peptide
TLLK

SEQ ID NO: 650 - protein, 4 aa, synthetic construct
  REGION 1..4: note = peptide
SLLK

SEQ ID NO: 651 - protein, 4 aa, synthetic construct
  REGION 1..4: note = peptide
IVLK

SEQ ID NO: 652 - protein, 4 aa, synthetic construct
  REGION 1..4: note = peptide
LTLK

SEQ ID NO: 653 - protein, 4 aa, synthetic construct
  REGION 1..4: note = peptide
LSLK

SEQ ID NO: 654 - protein, 4 aa, synthetic construct
  REGION 1..4: note = peptide
LALK

SEQ ID NO: 655 - protein, 4 aa, synthetic construct
  REGION 1..4: note = peptide
ITLK

SEQ ID NO: 656 - protein, 4 aa, synthetic construct
  REGION 1..4: note = peptide
ISLK

SEQ ID NO: 657 - protein, 4 aa, synthetic construct
  REGION 1..4: note = peptide
TVLK

SEQ ID NO: 658 - protein, 4 aa, synthetic construct
  REGION 1..4: note = peptide
SVLK

SEQ ID NO: 659 - protein, 4 aa, synthetic construct
  REGION 1..4: note = peptide
VTLK

SEQ ID NO: 660 - protein, 4 aa, synthetic construct
  REGION 1..4: note = peptide
VSLK

SEQ ID NO: 661 - protein, 4 aa, synthetic construct
  REGION 1..4: note = peptide
VLTK

SEQ ID NO: 662 - protein, 4 aa, synthetic construct
  REGION 1..4: note = peptide
TALK

SEQ ID NO: 663 - protein, 4 aa, synthetic construct
  REGION 1..4: note = peptide
SALK

SEQ ID NO: 664 - protein, 7 aa, synthetic construct
  REGION 1..7: note = peptide
KIAVLAI

SEQ ID NO: 665 - protein, 7 aa, synthetic construct
  REGION 1..7: note = peptide
KITVLAI

SEQ ID NO: 666 - protein, 7 aa, synthetic construct
  REGION 1..7: note = peptide
KIAVLTI

SEQ ID NO: 667 - protein, 7 aa, synthetic construct
  REGION 1..7: note = peptide
KIAVLSI

SEQ ID NO: 668 - protein, 7 aa, synthetic construct
  REGION 1..7: note = peptide
KISVLAI

SEQ ID NO: 669 - protein, 7 aa, synthetic construct
  REGION 1..7: note = peptide
KIATLAI

SEQ ID NO: 670 - protein, 7 aa, synthetic construct
  REGION 1..7: note = peptide
KIASLAI

SEQ ID NO: 671 - protein, 7 aa, synthetic construct
  REGION 1..7: note = peptide
KIASLSI

SEQ ID NO: 672 - protein, 7 aa, synthetic construct
  REGION 1..7: note = peptide
KTTVLAI

SEQ ID NO: 673 - protein, 7 aa, synthetic construct
  REGION 1..7: note = peptide
KSAVLAI

SEQ ID NO: 674 - protein, 7 aa, synthetic construct
  REGION 1..7: note = peptide
KIAVSAI

SEQ ID NO: 675 - protein, 7 aa, synthetic construct
  REGION 1..7: note = peptide
KSSVLAI

SEQ ID NO: 676 - protein, 7 aa, synthetic construct
  REGION 1..7: note = peptide
KTTTLAI

SEQ ID NO: 677 - protein, 7 aa, synthetic construct
  REGION 1..7: note = peptide
KIAVLTT

SEQ ID NO: 678 - protein, 7 aa, synthetic construct
  REGION 1..7: note = peptide
KIAVSSI

SEQ ID NO: 679 - protein, 7 aa, synthetic construct
  REGION 1..7: note = peptide
KIAVLAS

SEQ ID NO: 680 - protein, 7 aa, synthetic construct
  REGION 1..7: note = peptide
KSASLSI

SEQ ID NO: 681 - protein, 7 aa, synthetic construct
  REGION 1..7: note = peptide
KSSSLAI

SEQ ID NO: 682 - protein, 7 aa, synthetic construct
  REGION 1..7: note = peptide
KIAVTAT

SEQ ID NO: 683 - protein, 7 aa, synthetic construct
  REGION 1..7: note = peptide
KIAVTTT

SEQ ID NO: 684 - protein, 7 aa, synthetic construct
  REGION 1..7: note = peptide
KIAVSAS

SEQ ID NO: 685 - protein, 7 aa, synthetic construct
  REGION 1..7: note = peptide
KIAVSSS

SEQ ID NO: 686 - protein, 7 aa, synthetic construct
  REGION 1..7: note = peptide
KTAVTAT

SEQ ID NO: 687 - protein, 7 aa, synthetic construct
  REGION 1..7: note = peptide
KSAVSAS

SEQ ID NO: 688 - protein, 5 aa, synthetic construct
  REGION 1..5: note = peptide
TLVPR

SEQ ID NO: 689 - protein, 5 aa, synthetic construct
  REGION 1..5: note = peptide
SLVPR

SEQ ID NO: 690 - skipped

SEQ ID NO: 691 - protein, 5 aa, synthetic construct
  REGION 1..5: note = peptide
FTPVR